European Patent Specification EP 3 411 476 B1, published April 24, 2024. Title: Enhanced Production of Immunglobulins. Applicant: Trianni, Inc. The sequence listing filed with the application follows.

SEQUENCE LISTING (59 sequences)

SEQ ID NO: 1 - DNA, 55 bp, Homo sapiens
atggacatcagggctcctgctcagtttcttggcatcttgttgctctggtttccag

SEQ ID NO: 2 - DNA, 110 bp, Homo sapiens
gtaaaatgaactaaaatgggaatttcactgtaagtgttgacaggcatttggggactgtgttcttttatcatgcttacctttgtagatattcattatgtctccactcctag

SEQ ID NO: 3 - DNA, 23 bp, Homo sapiens
gtgccagatgtgacatccagatg

SEQ ID NO: 4 - DNA, 63 bp, Artificial Sequence
  Leader Exon1/Intron/Exon 2/TagsFLAG+Myc Tags
gactacaaggatgacgacgacaagggcagcggcgaacagaagctgatttcggaggaggacctg

SEQ ID NO: 5 - DNA, 46 bp, Homo sapiens
atgggatggagctgtatcatgctcttcttggcagcaacagctacag

SEQ ID NO: 6 - DNA, 82 bp, Homo sapiens
gtaaggggctcacagtagcaggcttgaggtctggacatatacatgggtgacaatgacatccactttgcctttctctccacag

SEQ ID NO: 7 - DNA, 23 bp, Homo sapiens
gtgtccactcccaggtccaactg

SEQ ID NO: 8 - DNA, 369 bp, Escherichia coli
ggtaccccagccgtgaccacctacaagctcgtcatcaacggaaagacgctcaagggcgaaaccactaccaaggcggtggatgccgaaaccgccgaaaaggccttcaagcagtacgctaacgacaatggggtggacggagtctggacgtacgatgatgccaccaagactttcaccgtgaccgaagtgaacactccggccgtcaccacttataagctcgtgatcaacgggaaaaccctgaagggagagactaccacaaaggccgtggatgctgagactgcagagaaggcgttcaaacagtacgccaacgacaacggcgtggacggcgtctggacctacgatgacgccactaagaccttcactgtgaccgaa

SEQ ID NO: 9 - DNA, 621 bp, Escherichia coli
atagatgaaattttagctgcattacctaagactgacacttacaaattaatccttaatggtaaaacattgaaaggcgaaacaactactgaagctgttgatgctgctactgcagaaaaagtcttcaaacaatacgctaacgacaacggtgttgacggtgaatggacttacgacgatgcgactaagacctttacagttactgaaaaaccagaagtgatcgatgcgtctgaattaacaccagccgtgacaacttacaaacttgttattaatggtaaaacattgaaaggcgaaacaactactgaagctgttgatgctgctactgcagaaaaagtcttcaaacaatacgctaacgacaacggtgttgacggtgaatggacttacgacgatgcgactaagacctttacagttactgaaaaaccagaagtgatcgatgcgtctgaattaacaccagccgtgacaacttacaaacttgttattaatggtaaaacattgaaaggcgaaacaactactaaagcagtagacgcagaaactgcagaaaaagccttcaaacaatacgctaacgacaacggtgttgatggtgtttggacttatgatgatgcgactaagacctttacggtaactgaa

SEQ ID NO: 10 - DNA, 741 bp, Escherichia coli
gtggataacaagttcaacaaggaacagcagaacgccttttacgagattctgcatctgcccaacctgaatgaggaacagcggaacgcattcattcagtctctgaaggatgatcctagccagtcggccaacctcctggctgaagcaaagaagctgaacgatgcccaagcgcccaaagtggacaacaagtttaacaaggagcagcagaatgctttctacgagatcctgcacctcccgaatctgaacgaggagcagagaaacgccttcatccaatcactgaaggacgacccgtcacagtccgccaaccttctggcggaagccaagaaactgaacgacgcccaggcgccaaaggtggacggatccgggtccggcagcggtaccccagccgtgaccacctacaagctcgtcatcaacggaaagacgctcaagggcgaaaccactaccaaggcggtggatgccgaaaccgccgaaaaggccttcaagcagtacgctaacgacaatggggtggacggagtctggacgtacgatgatgccaccaagactttcaccgtgaccgaagtgaacactccggccgtcaccacttataagctcgtgatcaacgggaaaaccctgaagggagagactaccacaaaggccgtggatgctgagactgcagagaaggcgttcaaacagtacgccaacgacaacggcgtggacggcgtctggacctacgatgacgccactaagaccttcactgtgaccgaa

SEQ ID NO: 11 - DNA, 1681 bp, Escherichia coli
aaacctcaacgccgatcagcgcaatggtttcattcagtccctgaaggacgatccgagccagtcagctaacgtgctcggggaggcccaaaagctgaatgactcccaggcgccgaaggccgacgcccagcaaaacaacttcaacaaggatcagcaatccgccttctatgaaatcctgaatatgcctaacctgaacgaagctcagcggaacgggttcatccagagccttaaggacgaccctagccagtccaccaacgtgctgggggaggccaagaaacttaacgaatcccaggccccgaaggcggacaacaactttaacaaggaacagcagaacgccttttacgagatcctcaacatgccgaacctcaacgaggaacagcgcaacggtttcatccagtccctgaaggacgatccatcccagtccgccaacctgttgagcgaggcgaagaagctgaatgagtcccaagcccccaaggctgacaacaagttcaataaggaacaacagaatgccttctacgaaattctgcacttgcccaatctgaacgaggagcagcgcaacggcttcatccaatctctgaaagacgacccgtcgcagtcggccaacttgctggccgaagccaagaagctcaacgacgctcaggcccctaaggccgacaacaagttcaacaaagagcaacagaacgcgttctacgagattctccacttgccgaacctgaccgaagaacaacggaacggattcattcagagcctgaaggatgacccttcggtgtcaaaggagatcctggcagaagccaaaaagctgaacgatgcccaggcaccaaaggaagaggacaacaacaagccgggcgacccgaggatctccgaagccactgatgggctgtccgattttctgaagtcacagactcctgctgaggacaccgtgaagtccatcgagctcgccgaggccaaggtgctggccaaccgggagctggataagtacggagtgtccgactactacaaaaacctgattaacaacgccaagactgtggaaggagtgaaggcattgatcgatgaaatcctggcggcgctcccaaaaaccgacacctacaaactgattctcaacggaaagacgctgaagggggaaactaccaccgaagcggtggacgccgccaccgccgaaaaggtgtttaagcagtatgctaacgacaacggtgtcgacggagagtggacctacgacgacgccactaagactttcaccgtgaccgagaagcccgaggtcatcgacgcgagcgagctcactcccgccgtgaccacctacaagctggtcatcaatggaaagactctgaagggcgaaactactactgaagccgtggatgcggcaaccgccgagaaagtgttcaagcaatacgcaaacgataacggggtggacggagagtggacctacgacgatgccacaaagaccttcaccgtcaccgaaaagcccgaagtgatcgacgcttccgaactgacgccggccgtgacaacttacaagctcgtcattaacggaaagacccttaagggcgaaaccacgaccaaggcagtggacgccgaaactgccgagaaggcgttcaagcagtacgccaacgacaacggcgtggacggagtgtggacttacgatgatgcgaccaagacgttcactgtgaccgagatggtcaccgaagtgccg

SEQ ID NO: 12 - DNA, 18 bp, Artificial Sequence
  Gly/Ser linker
ggatccggctccggatcc

SEQ ID NO: 13 - DNA, 45 bp, Artificial Sequence
  Gly/Ser linker
ggaggcggaggcagcggaggcggtggctcgggaggcggaggctcg

SEQ ID NO: 14 - DNA, 243 bp, Rattus rattus
gagatggtgtccaagccgatgatctactgggagtgttccaacgcgactctgacctgtgaagtgctggagggaaccgacgtggaactgaagctgtaccagggtaaagaacatctgcggtcgttgcgccaaaagaccatgagctaccagtggaccaacttgcgggcgcctttcaagtgcaaagccgtcaatagagtgtcccaggagagcgaaatggaggtcgtgaactgccccgaaaagggactg

SEQ ID NO: 15 - DNA, 561 bp, Rattus rattus
tcaacttccatcaccgcctacaagagcgagggagagagcgccgagttttccttccccctgaacctgggcgaagaaagcctccagggagaactgcgctggaaggcagaaaaggccccaagctctcagtcctggatcaccttcagcctgaagaaccagaaggtgtccgtgcagaagtccacttcaaacccgaagttccagctctccgaaaccctccctctgaccctgcaaatccctcaagtgtcgctgcaattcgcggggagcggaaatctgactctgactcttgaccggggcatcttgtaccaggaggtgaacctggtggtcatgaaggtgacccagcccgatagcaacaccctgacctgtgaagtgatgggacccacgtccccgaagatgcggctcattctgaagcaggagaaccaggaggctcgggtgtccagacaggaaaaggtcatccaagtgcaggccccggaagccggcgtgtggcagtgcctgctgtccgagggagaggaagtcaagatggactcgaaaatccaggtgctgtccaaagggctgaaccagactatg

SEQ ID NO: 16 - DNA, 1638 bp, Homo sapiens
gaaaggccttttccacctcatatccagctccctccagaaattcaagagtcccaggaagtcactctgacctgcttgctgaatttctcctgctatgggtatccgatccaattgcagtggctcctagagggggttccaatgaggcaggctgctgtcacctcgacctccttgaccatcaagtctgtcttcacccggagcgagctcaagttctccccacagtggagtcaccatgggaagattgtgacctgccagcttcaggatgcagatgggaagttcctctccaatgacacggtgcagctgaacgtgaagcacaccccgaagttggagatcaaggtcactcccagtgatgccatagtgagggagggggactctgtgaccatgacctgcgaggtcagcagcagcaacccggagtacacgacggtatcctggctcaaggatgggacctcgctgaagaagcagaatacattcacgctaaacctgcgcgaagtgaccaaggaccagagtgggaagtactgctgtcaggtctccaatgacgtgggcccgggaaggtcggaagaagtgttcctgcaagtgcagtatgccccggaaccttccacggttcagatcctccactcaccggctgtggagggaagtcaagtcgagtttctttgcatgtcactggccaatcctcttccaacaaattacacgtggtaccacaatgggaaagaaatgcagggaaggacagaggagaaagtccacatcccaaagatcctcccctggcacgctgggacttattcctgtgtggcagaaaacattcttggtactggacagaggggcccgggagctgagctggatgtccagtatcctcccaagaaggtgaccacagtgattcaaaaccccatgccgattcgagaaggagacacagtgaccctttcctgtaactacaattccagtaaccccagtgttacccggtatgaatggaaaccccatggcgcctgggaggagccatcgcttggggtgctgaagatccaaaacgttggctgggacaacacaaccatcgcctgcgcagcttgtaatagttggtgctcgtgggcctcccctgtcgccctgaatgtccagtatgccccccgagacgtgagggtccggaaaatcaagcccctttccgagattcactctggaaactcggtcagcctccaatgtgacttctcaagcagccaccccaaagaagtccagttcttctgggagaaaaatggcaggcttctggggaaagaaagccagctgaattttgactccatctccccagaagatgctgggagttacagctgctgggtgaacaactccataggacagacagcgtccaaggcctggacacttgaagtgctgtatgcacccaggaggctgcgtgtgtccatgagcccgggggaccaagtgatggaggggaagagtgcaaccctgacctgtgagagcgacgccaaccctcccgtctcccactacacctggtttgactggaataaccaaagcctcccctaccacagccagaagctgagattggagccggtgaaggtccagcactcgggtgcctactggtgccaggggaccaacagtgtgggcaagggccgttcgcctctcagcaccctcaccgtctactatagcccggagacc

SEQ ID NO: 17 - DNA, 120 bp, Homo sapiens
gcgcctggagcgctgccggccggtcatctgttgttgttcctgaccctgggggtgctgtcactgctgctgctcgtgaccggggcattcggtttccacctgtggagaaggcagtggcggtag

SEQ ID NO: 18 - DNA, 123 bp, Homo sapiens
cattcccggcaccgctacgcgctgattccgattcctctggccgtgatcaccacctgtatcgtgctctacatgaacggtatcctgaaatgcgacagaaagcccgacaggactaacagcaattag

SEQ ID NO: 19 - DNA, 99 bp, Rattus rattus
ccgctgtacctgatcgtgggggtgtcagccggcggtctgctgctcgtgttcttcggggcactgttcatcttctgcatttgcaagaggaagaagcggtag

SEQ ID NO: 20 - DNA, 288 bp, Homo sapiens
ccaccccgggcgtccgcactgccggcgccccctaccggaagcgcgctgcccgatccgcaaaccgccagcgccctgcctgacccgcccgcggctagcgccttgcctgccgcactggccgtgatttcattcctgctgggtctggggctcggggtggcctgcgtgttggcacggactcagatcaagaagctgtgctcctggagagacaaaaactccgccgcctgtgtggtgtacgaggacatgtcacactcgaggtgcaataccctgtcctcgccgaaccagtaccagtag

SEQ ID NO: 21 - protein, 23 aa, Homo sapiens
MGWSCIMLFLAATATGVHSQVQL

SEQ ID NO: 22 - protein, 21 aa, Artificial Sequence
  Leader Exon1/Intron/Exon 2/TagsFLAG+Myc Tags
DYKDDDDKGSGEQKLISEEDL

SEQ ID NO: 23 - protein, 26 aa, Homo sapiens
MDIRAPAQFLGILLLWFPGARCDIQM

SEQ ID NO: 24 - protein, 123 aa, Escherichia coli
GTPAVTTYKLVINGKTLKGETTTKAVDAETAEKAFKQYANDNGVDGVWTYDDATKTFTVTEVNTPAVTTYKLVINGKTLKGETTTKAVDAETAEKAFKQYANDNGVDGVWTYDDATKTFTVTE

SEQ ID NO: 25 - protein, 207 aa, Escherichia coli
IDEILAALPKTDTYKLILNGKTLKGETTTEAVDAATAEKVFKQYANDNGVDGEWTYDDATKTFTVTEKPEVIDASELTPAVTTYKLVINGKTLKGETTTEAVDAATAEKVFKQYANDNGVDGEWTYDDATKTFTVTEKPEVIDASELTPAVTTYKLVINGKTLKGETTTKAVDAETAEKAFKQYANDNGVDGVWTYDDATKTFTVTE

SEQ ID NO: 26 - protein, 247 aa, Escherichia coli
VDNKFNKEQQNAFYEILHLPNLNEEQRNAFIQSLKDDPSQSANLLAEAKKLNDAQAPKVDNKFNKEQQNAFYEILHLPNLNEEQRNAFIQSLKDDPSQSANLLAEAKKLNDAQAPKVDGSGSGSGTPAVTTYKLVINGKTLKGETTTKAVDAETAEKAFKQYANDNGVDGVWTYDDATKTFTVTEVNTPAVTTYKLVINGKTLKGETTTKAVDAETAEKAFKQYANDNGVDGVWTYDDATKTFTVTE

SEQ ID NO: 27 - protein, 581 aa, Escherichia coli
ANAAQHDEAQQNAFYQVLNMPNLNADQRNGFIQSLKDDPSQSANVLGEAQKLNDSQAPKADAQQNNFNKDQQSAFYEILNMPNLNEAQRNGFIQSLKDDPSQSTNVLGEAKKLNESQAPKADNNFNKEQQNAFYEILNMPNLNEEQRNGFIQSLKDDPSQSANLLSEAKKLNESQAPKADNKFNKEQQNAFYEILHLPNLNEEQRNGFIQSLKDDPSQSANLLAEAKKLNDAQAPKADNKFNKEQQNAFYEILHLPNLTEEQRNGFIQSLKDDPSVSKEILAEAKKLNDAQAPKEEDNNKPGDPRISEATDGLSDFLKSQTPAEDTVKSIELAEAKVLANRELDKYGVSDYYKNLINNAKTVEGVKALIDEILAALPKTDTYKLILNGKTLKGETTTEAVDAATAEKVFKQYANDNGVDGEWTYDDATKTFTVTEKPEVIDASELTPAVTTYKLVINGKTLKGETTTEAVDAATAEKVFKQYANDNGVDGEWTYDDATKTFTVTEKPEVIDASELTPAVTTYKLVINGKTLKGETTTKAVDAETAEKAFKQYANDNGVDGVWTYDDATKTFTVTEMVTEVP

SEQ ID NO: 28 - protein, 6 aa, Artificial Sequence
  Gly/Ser linker
GSGSGS

SEQ ID NO: 29 - protein, 15 aa, Artificial Sequence
  Gly/Ser Linker
GGGGSGGGGSGGGGS

SEQ ID NO: 30 - protein, 81 aa, Rattus rattus
EMVSKPMIYWECSNATLTCEVLEGTDVELKLYQGKEHLRSLRQKTMSYQWTNLRAPFKCKAVNRVSQESEMEVVNCPEKGL

SEQ ID NO: 31 - protein, 187 aa, Rattus rattus
STSITAYKSEGESAEFSFPLNLGEESLQGELRWKAEKAPSSQSWITFSLKNQKVSVQKSTSNPKFQLSETLPLTLQIPQVSLQFAGSGNLTLTLDRGILYQEVNLVVMKVTQPDSNTLTCEVMGPTSPKMRLILKQENQEARVSRQEKVIQVQAPEAGVWQCLLSEGEEVKMDSKIQVLSKGLNQTM

SEQ ID NO: 32 - protein, 80 aa, Homo sapiens
MKVTQPDSNTLTCEVMGPTSPKMRLILKQENQEARVSRQEKVIQVQAPEAGVWQCLLSEGEEVKMDSKIQVLSKGLNQTM

SEQ ID NO: 33 - protein, 39 aa, Homo sapiens
APGALPAGHLLLFLTLGVLSLLLLVTGAFGFHLWRRQWR

SEQ ID NO: 34 - protein, 40 aa, Homo sapiens
HSRHRYALIPIPLAVITTCIVLYMNGILKCDRKPDRTNSN

SEQ ID NO: 35 - protein, 32 aa, Rattus rattus
PLYLIVGVSAGGLLLVFFGALFIFCICKRKKR

SEQ ID NO: 36 - protein, 95 aa, Homo sapiens
PPRASALPAPPTGSALPDPQTASALPDPPAASALPAALAVISFLLGLGLGVACVLARTQIKKLCSWRDKNSAACVVYEDMSHSRCNTLSSPNQYQ

SEQ ID NO: 37 - DNA, 93 bp, Homo sapiens
gaattccttgaaaatggtgggacatccttatcagagaaaacagttcttctgctggtgactccatttctggcagcagcctggagccttcatccc

SEQ ID NO: 38 - protein, 31 aa, Homo sapiens
EFLENGGTSLSEKTVLLLVTPFLAAAWSLHP

SEQ ID NO: 39 - DNA, 90 bp, Homo sapiens
accaatgccacaacaaaggcagcagggggagcactccagtcaacagcaagtttgtttgtcgtgtcactgagtctcttgcatctttattca

SEQ ID NO: 40 - protein, 30 aa, Homo sapiens
TNATTKAAGGALQSTASLFVVSLSLLHLYS

SEQ ID NO: 41 - DNA, 96 bp, Homo sapiens
gtctcccaggtgaaaatttcaggagcccctaccctctccccatccctcctgggtttgctgctgcccgcctttggcattctcgtgtatctggagttc

SEQ ID NO: 42 - protein, 32 aa, Homo sapiens
VSQVKISGAPTLSPSLLGLLLPAFGILVYLEF

SEQ ID NO: 43 - DNA, 49 bp, Homo sapiens
atggaatcacagacccaggtcctcatgtttcttctgctctgggtatctg

SEQ ID NO: 44 - DNA, 199 bp, Homo sapiens
gtaagaaatttaaagtattaaaaccttttcaaagtttcatctttgtggtaagaaatttgcaatatgtgccagtgtgtaatatttcttacataataaatttgtgacagtatgataaggacatttaaatgaaaaatttcgactgttgttataatctatgtctgtgtatctatgaattttcactgcctattaattattacag

SEQ ID NO: 45 - DNA, 11 bp, Homo sapiens
gtgcctgtgca

SEQ ID NO: 46 - DNA, 324 bp, Homo sapiens
gacattcagatgacccagtctccatcctccatgtctgtgtctctgggagacacagtcactattacttgccgggcaagtcaggacgttgggatttatgtaaactggttccagcagaaaccagggaaatctcctaggcgtatgatttatcgtgcaacgaacttggcagatggggtcccatcaaggttcagcggcagtaggtctggatcagattattctctcaccatcagcagcctggagtctgaagatgtggcagactatcactgtctacagtatgatgagtatccattcacgttcggatccgggacgaagttggaaataaaacgg

SEQ ID NO: 47 - DNA, 45 bp, Homo sapiens; identical to SEQ ID NO: 13

SEQ ID NO: 48 - DNA, 348 bp, Homo sapiens
caggtacagctgaaagagtcaggacctggtctggtgcagccctcacagaccctgtctctcacctgcactgtctctggactctcattaatcagttatggtgtaagttgggctcgccagcctccagggaagggtctggagtggattgcagcaatatcaagtggtggaagcacatattataattcagttctcacatctcgactgagcatcagcagggacacctccaagagccaagttttcttaaaaatgaacagtctgcaaactgaagacacagccatttacttctgtaccagagaactctgggactactatgattactggggccaaggagtcatggtcacagtctcctca

SEQ ID NO: 49 - DNA, 696 bp, Rattus rattus
gctgaaacaacagcccccagaaacccgggaggtgattgcaagccttgtatatgtacaggctcagaagtatcatctgtcttcatcttccccccaaagcccaaagatgtgctcaccatcactctgactcctaaggtcacgtgtgttgtggtagacattagccaggacgatcccgaggtccatttcagctggtttgtagatgacgtggaagtccacacagctcagactcgaccaccagaggagcagttcaacagcactttccgctcagtcagtgaactccccatcctgcaccaggactggctcaatggcaggacgttcagatgcaaggtcaccagtgcagctttcccatcccccatcgagaaaaccatctccaaacccgaaggcagaacacaagttccgcatgtatacaccatgtcacctaccaaggaagagatgacccagaatgaagtcagtatcacctgcatggtaaaaggcttctatcccccagacatttatgtggagtggcagatgaacgggcagccacaggaaaactacaagaacactccacctacgatggacacagatgggagttacttcctctacagcaagctcaatgtgaagaaggaaaaatggcagcagggaaacacgttcacgtgttctgtgctgcatgaaggcctgcacaaccaccatactgagaagagtctctcccactcccccggt

SEQ ID NO: 50 - DNA, 124 bp, Mus musculus
aaagagcctcctccatccactgtctccaacatggcgaccgttgctgttctggttgtccttggagctgcaatagtcactggagctgtggtggcttttgtgatgaagatgagaaggagaaacacag

SEQ ID NO: 51 - DNA, 178 bp, Mus musculus
gtaggaaagggcagagtctgagttttctctcagcctcctttagagtgtgctctgctcatcaatggggaacacaggcacaccccacattgctactgtctctaactgggtctgctgtcagttctgggaacttcctagtgtcaagatcttcctggaactctcacagcttttcttctcacag

SEQ ID NO: 52 - DNA, 33 bp, Mus musculus
gtggaaaaggaggggactatgctctggctccag

SEQ ID NO: 53 - DNA, 172 bp, Mus musculus
gttagtgtggggacagagttgtcctggggacattggagtgaagttggagatgatgggagctctgggaatccataatagctcctccagagaaatcttctaggtgcctgagttgtgccatgaaatgaatatgtacatgtacatatgcatatacatttgttttgttttaccctag

SEQ ID NO: 54 - DNA, 83 bp, Mus musculus
gctcccagacctctgatctgtctctcccagattgtaaaggtgacactctagggtctgattggggaggggcaatgtggacatga

SEQ ID NO: 55 - protein, 20 aa, Homo sapiens
MESQTQVLMFLLLWVSGACA

SEQ ID NO: 56 - protein, 108 aa, Homo sapiens
DIQMTQSPSSMSVSLGDTVTITCRASQDVGIYVNWFQQKPGKSPRRMIYRATNLADGVPSRFSGSRSGSDYSLTISSLESEDVADYHCLQYDEYPFTFGSGTKLEIKR

SEQ ID NO: 57 - protein, 116 aa, Homo sapiens
QVQLKESGPGLVQPSQTLSLTCTVSGLSLISYGVSWARQPPGKGLEWIAAISSGGSTYYNSVLTSRLSISRDTSKSQVFLKMNSLQTEDTAIYFCTRELWDYYDYWGQGVMVTVSS

SEQ ID NO: 58 - protein, 232 aa, Rattus rattus
AETTAPRNPGGDCKPCICTGSEVSSVFIFPPKPKDVLTITLTPKVTCVVVDISQDDPEVHFSWFVDDVEVHTAQTRPPEEQFNSTFRSVSELPILHQDWLNGRTFRCKVTSAAFPSPIEKTISKPEGRTQVPHVYTMSPTKEEMTQNEVSITCMVKGFYPPDIYVEWQMNGQPQENYKNTPPTMDTDGSYFLYSKLNVKKEKWQQGNTFTCSVLHEGLHNHHTEKSLSHSPG

SEQ ID NO: 59 - protein, 79 aa, Mus musculus
KEPPPSTVSNMATVAVLVVLGAAIVTGAVVAFVMKMRRRNTGGKGGDYALAPGSQTSDLSLPDCKGDTLGSDWGGAMWT